European Patent Specification EP 3 221 340 B1, published May 22, 2024. Title: HNL binding agents and uses thereof. Applicant: KONINKL PHILIPS ELECTRONICS NV. The sequence listing filed with the application follows.

SEQUENCE LISTING (26 sequences)

SEQ ID NO: 1 - protein, 198 aa, Homo sapiens
MPLGLLWLGLALLGALHAQAQDSTSDLIPAPPLSKVPLQQNFQDNQFQGKWYVVGLAGNAILREDKDPQKMYATIYELKEDKSYNVTSVLFRKKKCDYWIRTFVPGCQPGEFTLGNIKSYPGLTSYLVRVVSTNYNQHAMVFFKKVSQNREYFKITLYGRTKELTSELKENFIRFSKSLGLPENHIVFPVPIDQCIDG

SEQ ID NO: 2 - protein, 116 aa, Mus musculus
DIVMTQTPATLSVTPGDSVSLSCRASQSIITDLHWYQQRSHESPRLLIKSASQSISGIPSRFSGSGSGTDFTLTINSVETEDFGMYFCQQSNSWPLTFGAGTKLELKRADAAPTVS

SEQ ID NO: 3 - protein, 116 aa, Mus musculus
VQLQESGPDLVAPSQSLSITCTVSGFSLSSYGVHWVRQPPGKGLEWLIVMWSDGSTTSNSALKSRLSISKDNSKSQVFLKVNSLQSDDTAIYYCARHYGYFTMDYWGQGTSVTVSS

SEQ ID NO: 4 - protein, 115 aa, Mus musculus
DIVLTQSTSSLSVSLGDRVTINCRASQDISNYLNWYQEKPDGTVKLLIYFTSRLHSGVPSRFSGSGSGTDYSLTITNLEQEDIATYFCQQGNTLPWTFGGGTKLEIKRADAAPTV

SEQ ID NO: 5 - protein, 118 aa, Mus musculus
EVQLEESGPGLVAPSQSLSITCTISGFSLTSYGIHWLRQPPGKDLEWLVVIWGDGSTTSNSALKSRLSISKDNSKSQVFFKMSGLQTDDTAIYYCARHRYSDYHAMDYWGPGTSVTVS

SEQ ID NO: 6 - protein, 115 aa, Mus musculus
DIVLTQTTSSLSVSLGDRVTINCRASQDISNYLNWYQEKPDGTVKLLIYFTSRLHSGVPSRFSGSGSGTDYSLTITNLEQEDIATYFCQQGNTLPWTFGGGTKLEIKRADAAPTV

SEQ ID NO: 7 - protein, 119 aa, Mus musculus
EVKLQESGPGLVAPSQSLSITCTISGFSLTSYGIHWLRQPPGKDLEWLVVIWGDGSTTSNSALKSRLSISKDNSKSQVFFKMSGLQTDDTAIYYCARHRYSDYHAMDYWGPGTSVTVSS

SEQ ID NO: 8 - protein, 11 aa, Mus musculus
RASQSIITDLH

SEQ ID NO: 9 - protein, 7 aa, Mus musculus
SASQSIS

SEQ ID NO: 10 - protein, 9 aa, Mus musculus
QQSNSWPLT

SEQ ID NO: 11 - protein, 10 aa, Mus musculus
GFSLSSYGVH

SEQ ID NO: 12 - protein, 16 aa, Mus musculus
VMWSDGSTTSNSALKS

SEQ ID NO: 13 - protein, 9 aa, Mus musculus
HYGYFTMDY

SEQ ID NO: 14 - protein, 11 aa, Mus musculus
RASQDISNYLN

SEQ ID NO: 15 - protein, 7 aa, Mus musculus
FTSRLHS

SEQ ID NO: 16 - protein, 11 aa, Mus musculus
HRYSDYHAMDY

SEQ ID NO: 17 - protein, 10 aa, Mus musculus
GFSLTSYGIH

SEQ ID NO: 18 - protein, 16 aa, Mus musculus
VIWGDGSTTSNSALKS

SEQ ID NO: 19 - protein, 11 aa, Mus musculus
HRYSDYHAMDY

SEQ ID NO: 20 - protein, 11 aa, Mus musculus
RASQDISNYLN

SEQ ID NO: 21 - protein, 7 aa, Mus musculus
FTSRLHS

SEQ ID NO: 22 - protein, 9 aa, Mus musculus
QQGNTLPWT

SEQ ID NO: 23 - protein, 10 aa, Mus musculus
GFSLTSYGIH

SEQ ID NO: 24 - protein, 16 aa, Mus musculus
VIWGDGSTTSNSALKS

SEQ ID NO: 25 - protein, 11 aa, Mus musculus
HRYSDYHAMDY

SEQ ID NO: 26 - protein, 72 aa, Homo sapiens
SYNVTSVLFRKKKCDYWIRTFVPGCQPGEFTLGNIKSYPGLTSYLVRVVSTNYNQHAMVFFKKVSQNREYFK